European Patent Specification EP 4 167 720 B1, published October 8, 2025. Title: POWDERY MILDEW RESISTANT GRAPEVINE PLANT. Applicant: FONDAZIONE EDMUND MACH SCIENZA BIOTECHNOLOGIES 4 B.V. The sequence listing filed with the application follows.

SEQUENCE LISTING (8 sequences)

SEQ ID NO: 1 - protein, 586 aa, Vitis vinifera
  WT protein Mlo13
MAGATGGRSLEQTPTWAVAVVCFVLVLISIIIEYIIHLTGKWLKKKHKRALYEALEKVKSELMLLGFISLLLTVGQGLISTICISKSVAATWHPCSKSEEEKSTTTEESDTESDNRRKLLSISGFGGGSRRVLAAAGEDKCSAKGQAPFVSSDAIHQLHIFIFVLAIFHVLYCILTLALGTAKMRRWKAWEKETRTVEYQFSHDPERFRFARETSFGRRHLSFWTNTPFLIWIVCFFRQFVRSVPKVDYFTLRHGFIMAHLAPQSHAKFDFQKYINRSLEEDFKVVVGISPPIWFFAVLFLLLNTHGWYSYLWLPFIPLIVILLVGTKLQVIITKMGLRIQERGEVVKGVPVVQLGDDLFWFNRPRLVLYLIHFVLFQNAFQLAFFAWTWYEFGFKSCFYAHTEDVVIRISMGVIIQILCSYVTLPLYALVTQMGSTMKPTIFHERVATALRNWHHTAKKNIKHNKHSGLATPMSSRPTTPSRGTSPAYLLRYYRSDMDSLQASPRRSNLDMEHWETDGSPSPSHPHHGDGSSSHHNQLHQGTSLEHDRDISAPSSSQVVPLPQPTLHQHEIDVVRKEFSFDRRER

SEQ ID NO: 2 - DNA, 1764 bp, Vitis vinifera
  WT cDNA Mlo13
atggctggggcaaccggaggaaggtcgctggagcagacgccgacatgggctgttgctgtagtttgttttgttttggtgttgatttctattatcattgagtacatcattcatctcactggaaagtggttgaagaagaaacacaagagagctctatatgaagcgctggaaaaggtcaaatcagagctaatgttgctagggttcatatccttgctcctaacagtaggacaaggtctgatatcgactatatgtatatcaaagagtgttgcagcaacttggcatccatgcagcaagtctgaagaagagaagagcacaacgactgaagaatcagacaccgaatccgataatagacgaaaacttctcagcatatcgggttttggtggaggcagccgacgcgttttggcggcagctggagaagacaaatgttcagctaagggtcaagccccatttgtgtcgtcggatgctattcaccaactgcacatattcatcttcgtactggccattttccatgtcctttactgcatcttaaccctggctttgggcacagctaagatgagaaggtggaaggcatgggaaaaggaaacaagaacagtcgagtaccagttctcccacgatccggagaggttcaggtttgccagggagacgtcttttggaagaaggcacttgagtttctggaccaatacaccctttctcatctggatagtatgtttcttcagacagttcgttaggtccgttccaaaagttgactacttcaccttaagacatggatttatcatggcacatttggcacctcaaagccatgcaaaatttgatttccaaaaatatatcaatagatcgctggaggaggatttcaaggtggttgtgggtatcagtccaccaatatggttctttgccgtgctattccttctcctcaacactcatggctggtactcttatctatggctgccattcatcccactgattgttatcctattggtgggaaccaagttacaggtgatcataaccaagatggggcttagaattcaagaaaggggagaggttgtgaagggagtgccggttgttcagcttggtgatgacctcttctggttcaatcgccctcgcctcgttctctacctcatccattttgtgctctttcagaacgcatttcagctggctttcttcgcatggacttggtatgaattcgggtttaagtcttgtttctatgcacacactgaagatgtggtgatcaggatttccatgggggtcatcatacagattctttgcagctacgtaactctcccgctctatgccctggtgacacagatgggttcaaccatgaagccaacgatcttccatgagagagtagccacggctctaaggaactggcaccacacggctaagaaaaacatcaaacacaacaagcattctgggctagccacacccatgtcaagtaggccaacaacgccttcccgcggcacgtcccctgcttacctcttgcgctactaccggagcgacatggacagcctccaagcatccccgagaaggtccaacttggacatggagcattgggagactgatgggtccccctccccctcgcacccgcaccatggtgacggctcatcctctcaccacaaccagctccaccaaggaacgtccttggaacatgatagagacatcagcgcgcctagctcctcccaagtggttcctcttccacaacccactctccaccaacacgaaatcgatgttgtgcgcaaggaattttcatttgatcgaagagagaggacgtga

SEQ ID NO: 3 - DNA, 1763 bp, Vitis vinifera
  cDNA Mlo13 1 bp deletion
atggctggggcaaccggaggaaggtcgctggagcagacgccgacatgggctgttgctgtagtttgttttgttttggtgttgatttctattatcattgagtacatcattcatctcactggaaagtggttgaagaagaaacacaagagagctctatatgaagcgctggaaaaggtcaaatcagagctaatgttgctagggttcatatccttgctcctaacagtaggacaaggtctgatatcgactatatgtatatcaaagagtgttgcagcaacttggcatccatgcagcaagtctgaagaagagaagagcacaacgactgaagaatcagacaccgaatccgataatagacgaaaacttctcagcatatcgggttttggtggaggcagccgacgcgttttggcggcagctggagaagacaaatgttcagctaagggtcaagccccatttgtgtcgtcggatgctattcaccaactgcacatattcatcttcgtactggccattttccatgtcctttactgcatcttaaccctggctttgggcacagctaagatgagaaggtggaaggcatgggaaaaggaaacaagaacagtcgagtaccagttctcccacgatccggagaggttcaggtttgccagggagacgtcttttggaagaaggcacttgagtttctggaccaatacaccctttctcatctggatagtatgtttcttcagacagttcgttaggtccgttccaaaagttgactacttcaccttaagacatggatttatcatggcacatttggcacctcaaagccatgcaaaatttgatttccaaaaatatatcaatagatcgctggaggaggatttcaaggtggttgtgggtatcagtccaccaatatggttctttgccgtgctattccttctcctcaacactcatggctggtactcttatctatggctgccattcatcccactgattgttatcctattggtgggaaccaagttacaggtgatcataaccaagatggggcttagaattcaagaaaggggagaggttgtgaagggagtgccggttgttcagcttggtgatgacctcttctggttcaatcgccctcgcctcgttctctacctcatccattttgtgctctttcagaacgcatttcagctggctttcttcgcatggacttggtatgaattcgggtttaagtcttgtttctatgcacacactgaagatgtggtgatcaggatttccatgggggtcatcatacagattctttgcagctacgtaactctcccgctctatgccctggtgacacagatgggttcaaccatgaagccaacgatcttccatgagagagtagccacggctctaaggaactggcaccacacggctaagaaaaacatcaaacacaacaagcattctgggctagccacacccatgtcaagtaggccaacacgccttcccgcggcacgtcccctgcttacctcttgcgctactaccggagcgacatggacagcctccaagcatccccgagaaggtccaacttggacatggagcattgggagactgatgggtccccctccccctcgcacccgcaccatggtgacggctcatcctctcaccacaaccagctccaccaaggaacgtccttggaacatgatagagacatcagcgcgcctagctcctcccaagtggttcctcttccacaacccactctccaccaacacgaaatcgatgttgtgcgcaaggaattttcatttgatcgaagagagaggacgtga

SEQ ID NO: 4 - DNA, 1761 bp, Vitis vinifera
  cDNA Mlo13 3 bp deletion
atggctggggcaaccggaggaaggtcgctggagcagacgccgacatgggctgttgctgtagtttgttttgttttggtgttgatttctattatcattgagtacatcattcatctcactggaaagtggttgaagaagaaacacaagagagctctatatgaagcgctggaaaaggtcaaatcagagctaatgttgctagggttcatatccttgctcctaacagtaggacaaggtctgatatcgactatatgtatatcaaagagtgttgcagcaacttggcatccatgcagcaagtctgaagaagagaagagcacaacgactgaagaatcagacaccgaatccgataatagacgaaaacttctcagcatatcgggttttggtggaggcagccgacgcgttttggcggcagctggagaagacaaatgttcagctaagggtcaagccccatttgtgtcgtcggatgctattcaccaactgcacatattcatcttcgtactggccattttccatgtcctttactgcatcttaaccctggctttgggcacagctaagatgagaaggtggaaggcatgggaaaaggaaacaagaacagtcgagtaccagttctcccacgatccggagaggttcaggtttgccagggagacgtcttttggaagaaggcacttgagtttctggaccaatacaccctttctcatctggatagtatgtttcttcagacagttcgttaggtccgttccaaaagttgactacttcaccttaagacatggatttatcatggcacatttggcacctcaaagccatgcaaaatttgatttccaaaaatatatcaatagatcgctggaggaggatttcaaggtggttgtgggtatcagtccaccaatatggttctttgccgtgctattccttctcctcaacactcatggctggtactcttatctatggctgccattcatcccactgattgttatcctattggtgggaaccaagttacaggtgatcataaccaagatggggcttagaattcaagaaaggggagaggttgtgaagggagtgccggttgttcagcttggtgatgacctcttctggttcaatcgccctcgcctcgttctctacctcatccattttgtgctctttcagaacgcatttcagctggctttcttcgcatggacttggtatgaattcgggtttaagtcttgtttctatgcacacactgaagatgtggtgatcaggatttccatgggggtcatcatacagattctttgcagctacgtaactctcccgctctatgccctggtgacacagatgggttcaaccatgaagccaacgatcttccatgagagagtagccacggctctaaggaactggcaccacacggctaagaaaaacatcaaacacaacaagcattctgggctagccacacccatgtcaagtaggccaacgccttcccgcggcacgtcccctgcttacctcttgcgctactaccggagcgacatggacagcctccaagcatccccgagaaggtccaacttggacatggagcattgggagactgatgggtccccctccccctcgcacccgcaccatggtgacggctcatcctctcaccacaaccagctccaccaaggaacgtccttggaacatgatagagacatcagcgcgcctagctcctcccaagtggttcctcttccacaacccactctccaccaacacgaaatcgatgttgtgcgcaaggaattttcatttgatcgaagagagaggacgtga

SEQ ID NO: 5 - DNA, 1765 bp, Vitis vinifera
  cDNA Mlo13 1 bp insertion
atggctggggcaaccggaggaaggtcgctggagcagacgccgacatgggctgttgctgtagtttgttttgttttggtgttgatttctattatcattgagtacatcattcatctcactggaaagtggttgaagaagaaacacaagagagctctatatgaagcgctggaaaaggtcaaatcagagctaatgttgctagggttcatatccttgctcctaacagtaggacaaggtctgatatcgactatatgtatatcaaagagtgttgcagcaacttggcatccatgcagcaagtctgaagaagagaagagcacaacgactgaagaatcagacaccgaatccgataatagacgaaaacttctcagcatatcgggttttggtggaggcagccgacgcgttttggcggcagctggagaagacaaatgttcagctaagggtcaagccccatttgtgtcgtcggatgctattcaccaactgcacatattcatcttcgtactggccattttccatgtcctttactgcatcttaaccctggctttgggcacagctaagatgagaaggtggaaggcatgggaaaaggaaacaagaacagtcgagtaccagttctcccacgatccggagaggttcaggtttgccagggagacgtcttttggaagaaggcacttgagtttctggaccaatacaccctttctcatctggatagtatgtttcttcagacagttcgttaggtccgttccaaaagttgactacttcaccttaagacatggatttatcatggcacatttggcacctcaaagccatgcaaaatttgatttccaaaaatatatcaatagatcgctggaggaggatttcaaggtggttgtgggtatcagtccaccaatatggttctttgccgtgctattccttctcctcaacactcatggctggtactcttatctatggctgccattcatcccactgattgttatcctattggtgggaaccaagttacaggtgatcataaccaagatggggcttagaattcaagaaaggggagaggttgtgaagggagtgccggttgttcagcttggtgatgacctcttctggttcaatcgccctcgcctcgttctctacctcatccattttgtgctctttcagaacgcatttcagctggctttcttcgcatggacttggtatgaattcgggtttaagtcttgtttctatgcacacactgaagatgtggtgatcaggatttccatgggggtcatcatacagattctttgcagctacgtaactctcccgctctatgccctggtgacacagatgggttcaaccatgaagccaacgatcttccatgagagagtagccacggctctaaggaactggcaccacacggctaagaaaaacatcaaacacaacaagcattctgggctagccacacccatgtcaagtaggccaacatacgccttcccgcggcacgtcccctgcttacctcttgcgctactaccggagcgacatggacagcctccaagcatccccgagaaggtccaacttggacatggagcattgggagactgatgggtccccctccccctcgcacccgcaccatggtgacggctcatcctctcaccacaaccagctccaccaaggaacgtccttggaacatgatagagacatcagcgcgcctagctcctcccaagtggttcctcttccacaacccactctccaccaacacgaaatcgatgttgtgcgcaaggaattttcatttgatcgaagagagaggacgtga

SEQ ID NO: 6 - protein, 587 aa, Vitis vinifera
  protein encoded by SEQ ID No. 3
MAGATGGRSLEQTPTWAVAVVCFVLVLISIIIEYIIHLTGKWLKKKHKRALYEALEKVKSELMLLGFISLLLTVGQGLISTICISKSVAATWHPCSKSEEEKSTTTEESDTESDNRRKLLSISGFGGGSRRVLAAAGEDKCSAKGQAPFVSSDAIHQLHIFIFVLAIFHVLYCILTLALGTAKMRRWKAWEKETRTVEYQFSHDPERFRFARETSFGRRHLSFWTNTPFLIWIVCFFRQFVRSVPKVDYFTLRHGFIMAHLAPQSHAKFDFQKYINRSLEEDFKVVVGISPPIWFFAVLFLLLNTHGWYSYLWLPFIPLIVILLVGTKLQVIITKMGLRIQERGEVVKGVPVVQLGDDLFWFNRPRLVLYLIHFVLFQNAFQLAFFAWTWYEFGFKSCFYAHTEDVVIRISMGVIIQILCSYVTLPLYALVTQMGSTMKPTIFHERVATALRNWHHTAKKNIKHNKHSGLATPMSSRPTRLPAARPLLTSCATTGATWTASKHPREGPTWTWSIGRLMGPPPPRTRTMVTAHPLTTTSSTKERPWNMIETSARLAPPKWFLFHNPLSTNTKSMLCARNFHLIEERGR

SEQ ID NO: 7 - protein, 586 aa, Vitis vinifera
  protein encoded by SEQ ID No. 4
MAGATGGRSLEQTPTWAVAVVCFVLVLISIIIEYIIHLTGKWLKKKHKRALYEALEKVKSELMLLGFISLLLTVGQGLISTICISKSVAATWHPCSKSEEEKSTTTEESDTESDNRRKLLSISGFGGGSRRVLAAAGEDKCSAKGQAPFVSSDAIHQLHIFIFVLAIFHVLYCILTLALGTAKMRRWKAWEKETRTVEYQFSHDPERFRFARETSFGRRHLSFWTNTPFLIWIVCFFRQFVRSVPKVDYFTLRHGFIMAHLAPQSHAKFDFQKYINRSLEEDFKVVVGISPPIWFFAVLFLLLNTHGWYSYLWLPFIPLIVILLVGTKLQVIITKMGLRIQERGEVVKGVPVVQLGDDLFWFNRPRLVLYLIHFVLFQNAFQLAFFAWTWYEFGFKSCFYAHTEDVVIRISMGVIIQILCSYVTLPLYALVTQMGSTMKPTIFHERVATALRNWHHTAKKNIKHNKHSGLATPMSSRPTPSRGTSPAYLLRYYRSDMDSLQASPRRSNLDMEHWETDGSPSPSHPHHGDGSSSHHNQLHQGTSLEHDRDISAPSSSQVVPLPQPTLHQHEIDVVRKEFSFDRRERT

SEQ ID NO: 8 - protein, 517 aa, Vitis vinifera
  protein encoded by SEQ ID No. 5
MAGATGGRSLEQTPTWAVAVVCFVLVLISIIIEYIIHLTGKWLKKKHKRALYEALEKVKSELMLLGFISLLLTVGQGLISTICISKSVAATWHPCSKSEEEKSTTTEESDTESDNRRKLLSISGFGGGSRRVLAAAGEDKCSAKGQAPFVSSDAIHQLHIFIFVLAIFHVLYCILTLALGTAKMRRWKAWEKETRTVEYQFSHDPERFRFARETSFGRRHLSFWTNTPFLIWIVCFFRQFVRSVPKVDYFTLRHGFIMAHLAPQSHAKFDFQKYINRSLEEDFKVVVGISPPIWFFAVLFLLLNTHGWYSYLWLPFIPLIVILLVGTKLQVIITKMGLRIQERGEVVKGVPVVQLGDDLFWFNRPRLVLYLIHFVLFQNAFQLAFFAWTWYEFGFKSCFYAHTEDVVIRISMGVIIQILCSYVTLPLYALVTQMGSTMKPTIFHERVATALRNWHHTAKKNIKHNKHSGLATPMSSRPTYAFPRHVPCLPLALLPERHGQPPSIPEKVQLGHGALGD